European Patent Application EP 4 501 352 A2, published February 5, 2025. Title: COMPOSITIONS AND METHODS FOR CAR T CELL THERAPY. Applicant: PURDUE RESEARCH FOUNDATION. Application EP. The sequence listing filed with the application follows.

SEQUENCE LISTING (3 sequences)

SEQ ID NO: 1 - DNA, 1554 bp, synthetic construct
  misc_feature 1..1554: note = Description of Artificial Sequence: Synthetic polynucleotide
  source 1..1554: mol_type = other DNA
atggccttaccagtgaccgccttgctcctgccgctggccttgctgctccacgccgccaggccggatgtcgtgatgacccagacccccctcagcctcccagtgtccctcggtgaccaggcttctattagttgcagatccagccagtccctcgtgcactctaacggtaatacctacctgagatggtatctccagaagcccggacagagccctaaggtgctgatctacaaagtctccaaccgggtgtctggagtccctgaccgcttctcagggagcggttccggcaccgacttcaccctgaagatcaaccgggtggaggccgaagacctcggcgtctatttctgctctcagagtacacatgtgccctggaccttcggcggagggaccaagctggagatcaaaagctccgcagacgatgccaagaaagatgccgctaagaaagacgatgctaagaaagacgatgcaaagaaagacggtggcgtgaagctggatgaaaccggaggaggtctcgtccagccaggaggagccatgaagctgagttgcgtgaccagcggattcacctttgggcactactggatgaactgggtgcgacagtccccagagaaggggctcgaatgggtcgctcagttcaggaacaaaccctacaattatgagacatactattcagacagcgtgaagggcaggtttactatcagtagagacgattccaaatctagcgtgtacctgcagatgaacaatctcagggtcgaagatacaggcatctactattgcacaggggcatcctatggtatggagtatctcggtcaggggacaagcgtcacagtcagtttcgtgccggtcttcctgccagcgaagcccaccacgacgccagcgccgcgaccaccaacaccggcgcccaccatcgcgtcgcagcccctgtccctgcgcccagaggcgtgccggccagcggcggggggcgcagtgcacacgagggggctggacttcgcctgtgatatctacatctgggcgcccttggccgggacttgtggggtccttctcctgtcactggttatcaccctttactgcaaccacaggaaccgtttctctgttgttaaacggggcagaaagaaactcctgtatatattcaaacaaccatttatgagaccagtacaaactactcaagaggaagatggctgtagctgccgatttccagaagaagaagaaggaggatgtgaactgagagtgaagttcagcaggagcgcagacgcccccgcgtaccagcagggccagaaccagctctataacgagctcaatctaggacgaagagaggagtacgatgttttggacaagagacgtggccgggaccctgagatggggggaaagccgagaaggaagaaccctcaggaaggcctgtacaatgaactgcagaaagataagatggcggaggcctacagtgagattgggatgaaaggcgagcgccggaggggcaaggggcacgatggcctttaccagggtctcagtacagccaccaaggacacctacgacgcccttcacatgcaggccctgccccctcgctaa

SEQ ID NO: 2 - protein, 517 aa, synthetic construct
  REGION 1..517: note = Description of Artificial Sequence: Synthetic polypeptide
MALPVTALLLPLALLLHAARPDVVMTQTPLSLPVSLGDQASISCRSSQSLVHSNGNTYLRWYLQKPGQSPKVLIYKVSNRVSGVPDRFSGSGSGTDFTLKINRVEAEDLGVYFCSQSTHVPWTFGGGTKLEIKSSADDAKKDAAKKDDAKKDDAKKDGGVKLDETGGGLVQPGGAMKLSCVTSGFTFGHYWMNWVRQSPEKGLEWVAQFRNKPYNYETYYSDSVKGRFTISRDDSKSSVYLQMNNLRVEDTGIYYCTGASYGMEYLGQGTSVTVSFVPVFLPAKPTTTPAPRPPTPAPTIASQPLSLRPEACRPAAGGAVHTRGLDFACDIYIWAPLAGTCGVLLLSLVITLYCNHRNRFSVVKRGRKKLLYIFKQPFMRPVQTTQEEDGCSCRFPEEEEGGCELRVKFSRSADAPAYQQGQNQLYNELNLGRREEYDVLDKRRGRDPEMGGKPRRKNPQEGLYNELQKDKMAEAYSEIGMKGERRRGKGHDGLYQGLSTATKDTYDALHMQALPPR

SEQ ID NO: 3 - DNA, 1560 bp, synthetic construct
  misc_feature 1..1560: note = Description of Artificial Sequence: Synthetic polynucleotide
  source 1..1560: mol_type = other DNA
gccaccatggccttaccagtgaccgccttgctcctgccgctggccttgctgctccacgccgccaggccggatgtcgtgatgacccagacccccctcagcctcccagtgtccctcggtgaccaggcttctattagttgcagatccagccagtccctcgtgcactctaacggtaatacctacctgagatggtatctccagaagcccggacagagccctaaggtgctgatctacaaagtctccaaccgggtgtctggagtccctgaccgcttctcagggagcggttccggcaccgacttcaccctgaagatcaaccgggtggaggccgaagacctcggcgtctatttctgctctcagagtacacatgtgccctggaccttcggcggagggaccaagctggagatcaaaagctccgcagacgatgccaagaaagatgccgctaagaaagacgatgctaagaaagacgatgcaaagaaagacggtggcgtgaagctggatgaaaccggaggaggtctcgtccagccaggaggagccatgaagctgagttgcgtgaccagcggattcacctttgggcactactggatgaactgggtgcgacagtccccagagaaggggctcgaatgggtcgctcagttcaggaacaaaccctacaattatgagacatactattcagacagcgtgaagggcaggtttactatcagtagagacgattccaaatctagcgtgtacctgcagatgaacaatctcagggtcgaagatacaggcatctactattgcacaggggcatcctatggtatggagtatctcggtcaggggacaagcgtcacagtcagtttcgtgccggtcttcctgccagcgaagcccaccacgacgccagcgccgcgaccaccaacaccggcgcccaccatcgcgtcgcagcccctgtccctgcgcccagaggcgtgccggccagcggcggggggcgcagtgcacacgagggggctggacttcgcctgtgatatctacatctgggcgcccttggccgggacttgtggggtccttctcctgtcactggttatcaccctttactgcaaccacaggaaccgtttctctgttgttaaacggggcagaaagaaactcctgtatatattcaaacaaccatttatgagaccagtacaaactactcaagaggaagatggctgtagctgccgatttccagaagaagaagaaggaggatgtgaactgagagtgaagttcagcaggagcgcagacgcccccgcgtaccagcagggccagaaccagctctataacgagctcaatctaggacgaagagaggagtacgatgttttggacaagagacgtggccgggaccctgagatggggggaaagccgagaaggaagaaccctcaggaaggcctgtacaatgaactgcagaaagataagatggcggaggcctacagtgagattgggatgaaaggcgagcgccggaggggcaaggggcacgatggcctttaccagggtctcagtacagccaccaaggacacctacgacgcccttcacatgcaggccctgccccctcgctaa